European Patent Application EP 4 147 712 A1, published March 15, 2023. Title: METHOD TO GENERATE A DOUBLE-STRANDED DNA POOL ENCODING NEOANTIGENS OF A TUMOR OF A PATIENT. Applicant: OncoDNA. The sequence listing filed with the application follows.

SEQUENCE LISTING (80 sequences)

SEQ ID NO: 1 - DNA, 25 bp, Artificial sequence
  T7 RNA Polymerase
taatacgactcactatagggataat

SEQ ID NO: 2 - DNA, 40 bp, Artificial sequence
  5' sequence element beta globin (translation enhancer)
acatttgcttctgacacaactgtgttcactagcaacctca

SEQ ID NO: 3 - DNA, 93 bp, Artificial sequence
  Endosomial Signal
atggcggcccccggcagcgcccggcgacccctgctgctgctactgctgttgctgctgctcggcctcatgcattgtgcgtcagcagcaatggac

SEQ ID NO: 4 - DNA, 81 bp, Artificial sequence
  Specific neoantigen sequence
gtcagtctggtcgtcagtggtcgggttgtagccgccaacaggggcctggtggcggcaggggacgctagaggtagggccgct

SEQ ID NO: 5 - DNA, 123 bp, Artificial sequence
  Sequence for presentation to T lymphocytes
  misc_feature (30)..(52): Sequence for sense/antisense pairing
tcgtctgactacacaattgtgcttcctgtgattggggccatcgtggttggtctctgccttatgggtatgggtgtctataaaatccgcctaaggtgtcaatcatctggataccagagaatctaa

SEQ ID NO: 6 - DNA, 134 bp, Artificial sequence
  Translation enhancer/mRNA stability
agctcgctttcttgctgtccaatttctattaaaggttcctttgttccctaagtccaactactaaactgggggatattatgaagggccttgagcatctggattctgcctaataaaaaactttattttcattgcaa

SEQ ID NO: 7 - DNA, 26 bp, Artificial sequence
  Forward primer
taatacgactcactatagggataata

SEQ ID NO: 8 - DNA, 297 bp, Artificial Sequence
  Reverse oligo
ttttttttttttttttttttttttttttttttttttttttttttttttttttttttttttttttttttttgcaatgaaaataaatgttttttattaggcagaatccagatgctcaaggcccttcataatatcccccagtttagtagttggacttagggaacaaaggaacctttaatagaaattggacagcaagaaagcgagctttagattctctggtatccagatgattgacaccttaggcggattttatagacacccatacccataaggcagagaccaaccacgatggccccaatc

SEQ ID NO: 9 - DNA, 174 bp, Artificial sequence
  Fused Seqs 4-5
  CDS (1)..(174)
atggcggcccccggcagcgcccggcgacccctgctgctgctactgctgttgctgctgctcggcctcatgcattgtgcgtcagcagcaatggacgtcagtctggtcgtcagtggtcgggttgtagccgccaacaggggcctggtggcggcaggggacgctagaggtagggccgct

SEQ ID NO: 10 - protein, 58 aa, Artificial sequence
  Synthetic Construct
MAAPGSARRPLLLLLLLLLLGLMHCASAAMDVSLVVSGRVVAANRGLVAAGDARGRAA

SEQ ID NO: 11 - DNA, 297 bp, Artificial sequence
  Fused Seqs. 3-5
  CDS (1)..(297)
atggcggcccccggcagcgcccggcgacccctgctgctgctactgctgttgctgctgctcggcctcatgcattgtgcgtcagcagcaatggacgtcagtctggtcgtcagtggtcgggttgtagccgccaacaggggcctggtggcggcaggggacgctagaggtagggccgcttcgtctgactacacaattgtgcttcctgtgattggggccatcgtggttggtctctgccttatgggtatgggtgtctataaaatccgcctaaggtgtcaatcatctggataccagagaatctaa

SEQ ID NO: 12 - protein, 98 aa, Artificial sequence
  Synthetic Construct
MAAPGSARRPLLLLLLLLLLGLMHCASAAMDVSLVVSGRVVAANRGLVAAGDARGRAASSDYTIVLPVIGAIVVGLCLMGMGVYKIRLRCQSSGYQRI

SEQ ID NO: 13 - DNA, 291 bp, Artificial Sequence
  F1OncoRNA
taatacgactcactatagggataatacatttgcttctgacacaactgtgttcactagcaacctcaatggcggcccccggcagcgcccggcgacccctgctgctgctactgctgttgctgctgctcggcctcatgcattgtgcgtcagcagcaatggacccgcgactcgttcctggttggaccaagcccattacgatcggttctcatgcgcatggtgatcaagtgggccaaggtggagaatcgtctgactacacaattgtgcttcctgtgattggggccatcgtggttggtc

SEQ ID NO: 14 - DNA, 291 bp, Artificial Sequence
  F2OncoRNA
taatacgactcactatagggataatacatttgcttctgacacaactgtgttcactagcaacctcaatggcggcccccggcagcgcccggcgacccctgctgctgctactgctgttgctgctgctcggcctcatgcattgtgcgtcagcagcaatggacgaggctgcacttttcggaaggtttaccatcaaaagcgatgtatggtcattccggatacttctgacagagctcattactaaatcgtctgactacacaattgtgcttcctgtgattggggccatcgtggttggtc

SEQ ID NO: 15 - DNA, 291 bp, Artificial Sequence
  F3OncoRNA
taatacgactcactatagggataatacatttgcttctgacacaactgtgttcactagcaacctcaatggcggcccccggcagcgcccggcgacccctgctgctgctactgctgttgctgctgctcggcctcatgcattgtgcgtcagcagcaatggacattgacttcgtattgtctaatgcaaggccggtcttgggtgttggaggggctgcaatgcttgggatagcaacgctcgctgtgtcgtctgactacacaattgtgcttcctgtgattggggccatcgtggttggtc

SEQ ID NO: 16 - DNA, 291 bp, Artificial Sequence
  F4OncoRNA
taatacgactcactatagggataatacatttgcttctgacacaactgtgttcactagcaacctcaatggcggcccccggcagcgcccggcgacccctgctgctgctactgctgttgctgctgctcggcctcatgcattgtgcgtcagcagcaatggacagacaacacagggatcgggatagagaaaaggaaagagaaaaagagaagggtaagccgaaaccgagatcacctcaaccactctcgtctgactacacaattgtgcttcctgtgattggggccatcgtggttggtc

SEQ ID NO: 17 - DNA, 291 bp, Artificial Sequence
  F5OncoRNA
taatacgactcactatagggataatacatttgcttctgacacaactgtgttcactagcaacctcaatggcggcccccggcagcgcccggcgacccctgctgctgctactgctgttgctgctgctcggcctcatgcattgtgcgtcagcagcaatggacaagcaacaagaggtacagttcaaatcatattacctgccaaaagatgatgagtattatcaattttgttatgtggacgaggactcgtctgactacacaattgtgcttcctgtgattggggccatcgtggttggtc

SEQ ID NO: 18 - DNA, 291 bp, Artificial Sequence
  F6OncoRNA
taatacgactcactatagggataatacatttgcttctgacacaactgtgttcactagcaacctcaatggcggcccccggcagcgcccggcgacccctgctgctgctactgctgttgctgctgctcggcctcatgcattgtgcgtcagcagcaatggacgtcgtatatttcactgctatgttcccatatgtggtactggtgatcctgctcataaggggggtaacccttcctggtgcaggatcgtctgactacacaattgtgcttcctgtgattggggccatcgtggttggtc

SEQ ID NO: 19 - DNA, 291 bp, Artificial Sequence
  F6OncoRNA
taatacgactcactatagggataatacatttgcttctgacacaactgtgttcactagcaacctcaatggcggcccccggcagcgcccggcgacccctgctgctgctactgctgttgctgctgctcggcctcatgcattgtgcgtcagcagcaatggacgccggggacgctcccacatttcccaggccttccggaccacgcaatactctctggcaagaactcccagccgtccaagccagctcgtctgactacacaattgtgcttcctgtgattggggccatcgtggttggtc

SEQ ID NO: 20 - DNA, 291 bp, Artificial Sequence
  F8OncoRNA
taatacgactcactatagggataatacatttgcttctgacacaactgtgttcactagcaacctcaatggcggcccccggcagcgcccggcgacccctgctgctgctactgctgttgctgctgctcggcctcatgcattgtgcgtcagcagcaatggaccataatctcattgcggaagttggagcccccgcggcgctgggcgtgagaggggcccttgagggattgccacggccccccccatcgtctgactacacaattgtgcttcctgtgattggggccatcgtggttggtc

SEQ ID NO: 21 - DNA, 291 bp, Artificial Sequence
  F9OncoRNA
taatacgactcactatagggataatacatttgcttctgacacaactgtgttcactagcaacctcaatggcggcccccggcagcgcccggcgacccctgctgctgctactgctgttgctgctgctcggcctcatgcattgtgcgtcagcagcaatggacaacatcccccgactggtcccaggctggaccaaaccgattactatcgggtcccatgctcatggtgaccaagtaggacaagggtcgtctgactacacaattgtgcttcctgtgattggggccatcgtggttggtc

SEQ ID NO: 22 - DNA, 291 bp, Artificial Sequence
  F10OncoRNA
taatacgactcactatagggataatacatttgcttctgacacaactgtgttcactagcaacctcaatggcggcccccggcagcgcccggcgacccctgctgctgctactgctgttgctgctgctcggcctcatgcattgtgcgtcagcagcaatggactgcctgcaagactggggtccattcttctcactcgccgtgcctagtatgcttatgatctgtttcgagtggtgggcttacgagtcgtctgactacacaattgtgcttcctgtgattggggccatcgtggttggtc

SEQ ID NO: 23 - DNA, 291 bp, Artificial Sequence
  F11OncoRNA
taatacgactcactatagggataatacatttgcttctgacacaactgtgttcactagcaacctcaatggcggcccccggcagcgcccggcgacccctgctgctgctactgctgttgctgctgctcggcctcatgcattgtgcgtcagcagcaatggactttgtgctcagcaacgccaggccggtcctcggcgtgggtggagctgcgatgctcggcattgccaccttggcggtgaagcggtcgtctgactacacaattgtgcttcctgtgattggggccatcgtggttggtc

SEQ ID NO: 24 - DNA, 291 bp, Artificial Sequence
  F12OncoRNA
taatacgactcactatagggataatacatttgcttctgacacaactgtgttcactagcaacctcaatggcggcccccggcagcgcccggcgacccctgctgctgctactgctgttgctgctgctcggcctcatgcattgtgcgtcagcagcaatggacgccattacaagagctgagagcttttctgtcatgtatgccccctttgctactaagatccgagcagacaaaatagagaaggtctcgtctgactacacaattgtgcttcctgtgattggggccatcgtggttggtc

SEQ ID NO: 25 - DNA, 291 bp, Artificial Sequence
  F13OncoRNA
taatacgactcactatagggataatacatttgcttctgacacaactgtgttcactagcaacctcaatggcggcccccggcagcgcccggcgacccctgctgctgctactgctgttgctgctgctcggcctcatgcattgtgcgtcagcagcaatggacggatggaagaccacctgtgaatactacaccttcatgtgggttaccctccccatcgacctgaacaataaatcagcgaaacaatcgtctgactacacaattgtgcttcctgtgattggggccatcgtggttggtc

SEQ ID NO: 26 - DNA, 291 bp, Artificial Sequence
  F14OncoRNA
taatacgactcactatagggataatacatttgcttctgacacaactgtgttcactagcaacctcaatggcggcccccggcagcgcccggcgacccctgctgctgctactgctgttgctgctgctcggcctcatgcattgtgcgtcagcagcaatggactgggaggaatttactgatcaactgtcattcatcggaagaataaggccgttggccgaaaaaacgggcatttgcaaaatccgatcgtctgactacacaattgtgcttcctgtgattggggccatcgtggttggtc

SEQ ID NO: 27 - DNA, 291 bp, Artificial Sequence
  F15OncoRNA
taatacgactcactatagggataatacatttgcttctgacacaactgtgttcactagcaacctcaatggcggcccccggcagcgcccggcgacccctgctgctgctactgctgttgctgctgctcggcctcatgcattgtgcgtcagcagcaatggaccttcccggcatcggtcatgcgtgtggtcacaatctgatagcggaggtcggtgctccagccgcacttggtgtccgaggagcctcgtctgactacacaattgtgcttcctgtgattggggccatcgtggttggtc

SEQ ID NO: 28 - DNA, 291 bp, Artificial Sequence
  F16OncoRNA
taatacgactcactatagggataatacatttgcttctgacacaactgtgttcactagcaacctcaatggcggcccccggcagcgcccggcgacccctgctgctgctactgctgttgctgctgctcggcctcatgcattgtgcgtcagcagcaatggacttctcagaggacggagaatatttcgcttatggggtctcagcatcagggtccgattgggtaacgataaaatttatgaaagtttcgtctgactacacaattgtgcttcctgtgattggggccatcgtggttggtc

SEQ ID NO: 29 - DNA, 291 bp, Artificial Sequence
  F17OncoRNA
taatacgactcactatagggataatacatttgcttctgacacaactgtgttcactagcaacctcaatggcggcccccggcagcgcccggcgacccctgctgctgctactgctgttgctgctgctcggcctcatgcattgtgcgtcagcagcaatggactgtggtggcggtatccagacccgcgaagtttattgcgcccaatccctcccggctgcagccgctctgagggctaaggaggtttcgtctgactacacaattgtgcttcctgtgattggggccatcgtggttggtc

SEQ ID NO: 30 - DNA, 291 bp, Artificial Sequence
  F18OncoRNA
taatacgactcactatagggataatacatttgcttctgacacaactgtgttcactagcaacctcaatggcggcccccggcagcgcccggcgacccctgctgctgctactgctgttgctgctgctcggcctcatgcattgtgcgtcagcagcaatggaccccgacgctatgcttctggcggaaattcgctcagttggccagacggaatacaacgggttccacctgtccaaaaagatagtctcgtctgactacacaattgtgcttcctgtgattggggccatcgtggttggtc

SEQ ID NO: 31 - DNA, 291 bp, Artificial Sequence
  F19OncoRNA
taatacgactcactatagggataatacatttgcttctgacacaactgtgttcactagcaacctcaatggcggcccccggcagcgcccggcgacccctgctgctgctactgctgttgctgctgctcggcctcatgcattgtgcgtcagcagcaatggacagctccggcaagcttctcgctaaaaccgtatatctgcgggaggcggaggggatgtttgacatacacattgtacaaaacccgtcgtctgactacacaattgtgcttcctgtgattggggccatcgtggttggtc

SEQ ID NO: 32 - DNA, 291 bp, Artificial Sequence
  F20OncoRNA
taatacgactcactatagggataatacatttgcttctgacacaactgtgttcactagcaacctcaatggcggcccccggcagcgcccggcgacccctgctgctgctactgctgttgctgctgctcggcctcatgcattgtgcgtcagcagcaatggacagcgtacccggcgcggtgcttatggacattaagtcagagcttttgaggtatgagatacagttcaaaggcaatgcacacacatcgtctgactacacaattgtgcttcctgtgattggggccatcgtggttggtc

SEQ ID NO: 33 - DNA, 291 bp, Artificial Sequence
  F21OncoRNA
taatacgactcactatagggataatacatttgcttctgacacaactgtgttcactagcaacctcaatggcggcccccggcagcgcccggcgacccctgctgctgctactgctgttgctgctgctcggcctcatgcattgtgcgtcagcagcaatggactctaaacaagaaggcttcatagacacggccctgcgaaagtacgtcgaaaacctggtgttgcatgggattcctatggcatcatcgtctgactacacaattgtgcttcctgtgattggggccatcgtggttggtc

SEQ ID NO: 34 - DNA, 291 bp, Artificial Sequence
  F22OncoRNA
taatacgactcactatagggataatacatttgcttctgacacaactgtgttcactagcaacctcaatggcggcccccggcagcgcccggcgacccctgctgctgctactgctgttgctgctgctcggcctcatgcattgtgcgtcagcagcaatggacataatgaaccatgctgacagtgctacaggaaaggtcaagatagaacgggagggggtcttttacccgcttttgctgcaaagctcgtctgactacacaattgtgcttcctgtgattggggccatcgtggttggtc

SEQ ID NO: 35 - DNA, 291 bp, Artificial Sequence
  F23OncoRNA
taatacgactcactatagggataatacatttgcttctgacacaactgtgttcactagcaacctcaatggcggcccccggcagcgcccggcgacccctgctgctgctactgctgttgctgctgctcggcctcatgcattgtgcgtcagcagcaatggacgcgagcccgagcaacttgaaaggcaagaccgagatcttcgctcacgtagaactgagagttatgcagggactgtatatagattcgtctgactacacaattgtgcttcctgtgattggggccatcgtggttggtc

SEQ ID NO: 36 - DNA, 291 bp, Artificial Sequence
  F24OncoRNA
taatacgactcactatagggataatacatttgcttctgacacaactgtgttcactagcaacctcaatggcggcccccggcagcgcccggcgacccctgctgctgctactgctgttgctgctgctcggcctcatgcattgtgcgtcagcagcaatggacgaagctggagtaggttttttgagcaaggatcgaaagattgctctttatttgacgaatgaacaccaggtctcaatgcccatctcgtctgactacacaattgtgcttcctgtgattggggccatcgtggttggtc

SEQ ID NO: 37 - DNA, 291 bp, Artificial Sequence
  F25OncoRNA
taatacgactcactatagggataatacatttgcttctgacacaactgtgttcactagcaacctcaatggcggcccccggcagcgcccggcgacccctgctgctgctactgctgttgctgctgctcggcctcatgcattgtgcgtcagcagcaatggacagtatgctcagattttataataaaggcgttaagggaccccttgaagcgagcgatactgttgaacacgcactcattcaaatatcgtctgactacacaattgtgcttcctgtgattggggccatcgtggttggtc

SEQ ID NO: 38 - DNA, 291 bp, Artificial Sequence
  F26OncoRNA
taatacgactcactatagggataatacatttgcttctgacacaactgtgttcactagcaacctcaatggcggcccccggcagcgcccggcgacccctgctgctgctactgctgttgctgctgctcggcctcatgcattgtgcgtcagcagcaatggacgtctttccactggaggagcagatgggaaaaataacacgagatggcagttaccatatcgcagttctcgcgaattccaagctctcgtctgactacacaattgtgcttcctgtgattggggccatcgtggttggtc

SEQ ID NO: 39 - DNA, 291 bp, Artificial Sequence
  F27OncoRNA
taatacgactcactatagggataatacatttgcttctgacacaactgtgttcactagcaacctcaatggcggcccccggcagcgcccggcgacccctgctgctgctactgctgttgctgctgctcggcctcatgcattgtgcgtcagcagcaatggactccgagctctacaagagggcgggcaagatgaatacggttggtctctcacaagaagcgatactgatcgatccgtttcacgtgtcgtctgactacacaattgtgcttcctgtgattggggccatcgtggttggtc

SEQ ID NO: 40 - DNA, 291 bp, Artificial Sequence
  F28OncoRNA
taatacgactcactatagggataatacatttgcttctgacacaactgtgttcactagcaacctcaatggcggcccccggcagcgcccggcgacccctgctgctgctactgctgttgctgctgctcggcctcatgcattgtgcgtcagcagcaatggactcccttctggggctgaaacagatttctccagtggatagggcagccatggagatttataacgtttttcacgggaaaacagagtcgtctgactacacaattgtgcttcctgtgattggggccatcgtggttggtc

SEQ ID NO: 41 - DNA, 291 bp, Artificial Sequence
  F29OncoRNA
taatacgactcactatagggataatacatttgcttctgacacaactgtgttcactagcaacctcaatggcggcccccggcagcgcccggcgacccctgctgctgctactgctgttgctgctgctcggcctcatgcattgtgcgtcagcagcaatggacattgtaacagcgggtagaccccaccttcttgagatgttgaactcagtccaattcgctggcgagagtaaatacaaaatcgactcgtctgactacacaattgtgcttcctgtgattggggccatcgtggttggtc

SEQ ID NO: 42 - DNA, 291 bp, Artificial Sequence
  F30OncoRNA
taatacgactcactatagggataatacatttgcttctgacacaactgtgttcactagcaacctcaatggcggcccccggcagcgcccggcgacccctgctgctgctactgctgttgctgctgctcggcctcatgcattgtgcgtcagcagcaatggacgtggctcacgggagcgagcaaacagaaatccccttttactctggactcgttaacattgatttggcaaaactcaaacggatgtcgtctgactacacaattgtgcttcctgtgattggggccatcgtggttggtc

SEQ ID NO: 43 - DNA, 291 bp, Artificial Sequence
  F31OncoRNA
taatacgactcactatagggataatacatttgcttctgacacaactgtgttcactagcaacctcaatggcggcccccggcagcgcccggcgacccctgctgctgctactgctgttgctgctgctcggcctcatgcattgtgcgtcagcagcaatggaccagtacctctcacccatggtacatattctgggacttgagagggtggcaaagaatactgaaaaattcgccggtatatctgattcgtctgactacacaattgtgcttcctgtgattggggccatcgtggttggtc

SEQ ID NO: 44 - DNA, 291 bp, Artificial Sequence
  F32OncoRNA
taatacgactcactatagggataatacatttgcttctgacacaactgtgttcactagcaacctcaatggcggcccccggcagcgcccggcgacccctgctgctgctactgctgttgctgctgctcggcctcatgcattgtgcgtcagcagcaatggacatgtcccaggttatagagatcaaaaatcgggcacttgctgggcactttaccgattatttggaaggcgtaagtaagcccctttcgtctgactacacaattgtgcttcctgtgattggggccatcgtggttggtc

SEQ ID NO: 45 - DNA, 291 bp, Artificial Sequence
  F33OncoRNA
taatacgactcactatagggataatacatttgcttctgacacaactgtgttcactagcaacctcaatggcggcccccggcagcgcccggcgacccctgctgctgctactgctgttgctgctgctcggcctcatgcattgtgcgtcagcagcaatggacatgcttgcaatctctcttcgggggtatccttcaggggctgtgcacattaacaccgaggttgaacagaagttgaaggatttttcgtctgactacacaattgtgcttcctgtgattggggccatcgtggttggtc

SEQ ID NO: 46 - DNA, 291 bp, Artificial Sequence
  F34OncoRNA
taatacgactcactatagggataatacatttgcttctgacacaactgtgttcactagcaacctcaatggcggcccccggcagcgcccggcgacccctgctgctgctactgctgttgctgctgctcggcctcatgcattgtgcgtcagcagcaatggacgttgagcctctttcattgttcaagaaaaatcttggctacagaacgatccagcatgctatggcagactcagaggtaattggttcgtctgactacacaattgtgcttcctgtgattggggccatcgtggttggtc

SEQ ID NO: 47 - DNA, 291 bp, Artificial Sequence
  F35OncoRNA
taatacgactcactatagggataatacatttgcttctgacacaactgtgttcactagcaacctcaatggcggcccccggcagcgcccggcgacccctgctgctgctactgctgttgctgctgctcggcctcatgcattgtgcgtcagcagcaatggactcaaaggtgaaagtacttaacatcagcgaactccatggctatgagtttcaggcaatgggtacgcgagaccccgctatactttcgtctgactacacaattgtgcttcctgtgattggggccatcgtggttggtc

SEQ ID NO: 48 - DNA, 291 bp, Artificial Sequence
  F36OncoRNA
taatacgactcactatagggataatacatttgcttctgacacaactgtgttcactagcaacctcaatggcggcccccggcagcgcccggcgacccctgctgctgctactgctgttgctgctgctcggcctcatgcattgtgcgtcagcagcaatggaccacaagaaactggccttgatcggaccaaaccaggatgtccgaatgacactctcaggatttgaggctagtgtagaaatctattcgtctgactacacaattgtgcttcctgtgattggggccatcgtggttggtc

SEQ ID NO: 49 - DNA, 291 bp, Artificial Sequence
  F37OncoRNA
taatacgactcactatagggataatacatttgcttctgacacaactgtgttcactagcaacctcaatggcggcccccggcagcgcccggcgacccctgctgctgctactgctgttgctgctgctcggcctcatgcattgtgcgtcagcagcaatggaccctggtcacgcttcttttgtcatggcgtatatccaagaacggttgaaagtgaataccaaactcttggacggtatttccgaatcgtctgactacacaattgtgcttcctgtgattggggccatcgtggttggtc

SEQ ID NO: 50 - DNA, 291 bp, Artificial Sequence
  F38OncoRNA
taatacgactcactatagggataatacatttgcttctgacacaactgtgttcactagcaacctcaatggcggcccccggcagcgcccggcgacccctgctgctgctactgctgttgctgctgctcggcctcatgcattgtgcgtcagcagcaatggacaaggatgtaatagagtcagtgaaggccttgagcatcaatcgatataccctgtttggtgctcagatgcatgaacctttgggctcgtctgactacacaattgtgcttcctgtgattggggccatcgtggttggtc

SEQ ID NO: 51 - DNA, 291 bp, Artificial Sequence
  F39OncoRNA
taatacgactcactatagggataatacatttgcttctgacacaactgtgttcactagcaacctcaatggcggcccccggcagcgcccggcgacccctgctgctgctactgctgttgctgctgctcggcctcatgcattgtgcgtcagcagcaatggaccagcacgtgcgggccataaagaagttcgaaatcctgatgtactcctccggcaacacacccgtggagggggcccttctcgactcgtctgactacacaattgtgcttcctgtgattggggccatcgtggttggtc

SEQ ID NO: 52 - DNA, 291 bp, Artificial Sequence
  F40OncoRNA
taatacgactcactatagggataatacatttgcttctgacacaactgtgttcactagcaacctcaatggcggcccccggcagcgcccggcgacccctgctgctgctactgctgttgctgctgctcggcctcatgcattgtgcgtcagcagcaatggacggggtctcaactgatcgcattaaaatggagcaatatcttctctttgaaagtaacggcaaacacttggttattcccgcagcatcgtctgactacacaattgtgcttcctgtgattggggccatcgtggttggtc

SEQ ID NO: 53 - DNA, 291 bp, Artificial Sequence
  F41OncoRNA
taatacgactcactatagggataatacatttgcttctgacacaactgtgttcactagcaacctcaatggcggcccccggcagcgcccggcgacccctgctgctgctactgctgttgctgctgctcggcctcatgcattgtgcgtcagcagcaatggacacaataaaggattactctaggagccatttgaaggggatgcccctcttcgctgtcatcgtactggagcaggagaacgcggggtcgtctgactacacaattgtgcttcctgtgattggggccatcgtggttggtc

SEQ ID NO: 54 - DNA, 291 bp, Artificial Sequence
  F42OncoRNA
taatacgactcactatagggataatacatttgcttctgacacaactgtgttcactagcaacctcaatggcggcccccggcagcgcccggcgacccctgctgctgctactgctgttgctgctgctcggcctcatgcattgtgcgtcagcagcaatggacatgatagagcaagatgttgcggaaattggtctgcgactcgcctataaggtgtccagccctactctccactttaacggtaagtcgtctgactacacaattgtgcttcctgtgattggggccatcgtggttggtc

SEQ ID NO: 55 - DNA, 291 bp, Artificial Sequence
  F43OncoRNA
taatacgactcactatagggataatacatttgcttctgacacaactgtgttcactagcaacctcaatggcggcccccggcagcgcccggcgacccctgctgctgctactgctgttgctgctgctcggcctcatgcattgtgcgtcagcagcaatggactacaaattgcagaggcatatcgacaaagaaggtacaaatcttgggttcatggttgcccttcccgagtctgtgatagcaagttcgtctgactacacaattgtgcttcctgtgattggggccatcgtggttggtc

SEQ ID NO: 56 - DNA, 291 bp, Artificial Sequence
  F44OncoRNA
taatacgactcactatagggataatacatttgcttctgacacaactgtgttcactagcaacctcaatggcggcccccggcagcgcccggcgacccctgctgctgctactgctgttgctgctgctcggcctcatgcattgtgcgtcagcagcaatggacataatgcacgcagtacaaaaaacacttattctgcgggaacccaagaacgacctcagctacggggaggggagtgcagtattctcgtctgactacacaattgtgcttcctgtgattggggccatcgtggttggtc

SEQ ID NO: 57 - DNA, 291 bp, Artificial Sequence
  F45OncoRNA
taatacgactcactatagggataatacatttgcttctgacacaactgtgttcactagcaacctcaatggcggcccccggcagcgcccggcgacccctgctgctgctactgctgttgctgctgctcggcctcatgcattgtgcgtcagcagcaatggacaaggccccggcagaaaatatgacgaaatactcaggtcatagaggggtcagcgaactttttcaagacgtcctgatactcatttcgtctgactacacaattgtgcttcctgtgattggggccatcgtggttggtc

SEQ ID NO: 58 - DNA, 291 bp, Artificial Sequence
  F46OncoRNA
taatacgactcactatagggataatacatttgcttctgacacaactgtgttcactagcaacctcaatggcggcccccggcagcgcccggcgacccctgctgctgctactgctgttgctgctgctcggcctcatgcattgtgcgtcagcagcaatggacgccgtttcccatctcggcgaaagatatcaaggaaccgccaaaatcatgagtcctttgctgtttaataaggacgttgagatctcgtctgactacacaattgtgcttcctgtgattggggccatcgtggttggtc

SEQ ID NO: 59 - DNA, 291 bp, Artificial Sequence
  F47OncoRNA
taatacgactcactatagggataatacatttgcttctgacacaactgtgttcactagcaacctcaatggcggcccccggcagcgcccggcgacccctgctgctgctactgctgttgctgctgctcggcctcatgcattgtgcgtcagcagcaatggacgagcccgcactcgacacattggagtatatgagtcttcacaaaggtaaaaacgtcttccaaagtgcgggcatccgcgtgatatcgtctgactacacaattgtgcttcctgtgattggggccatcgtggttggtc

SEQ ID NO: 60 - DNA, 291 bp, Artificial Sequence
  F48OncoRNA
taatacgactcactatagggataatacatttgcttctgacacaactgtgttcactagcaacctcaatggcggcccccggcagcgcccggcgacccctgctgctgctactgctgttgctgctgctcggcctcatgcattgtgcgtcagcagcaatggacttcgatatgaacaaaaaattgatccaccagtatgagacaccctccgccggtatccgcttggtcgtagaggggtcagcgctttcgtctgactacacaattgtgcttcctgtgattggggccatcgtggttggtc

SEQ ID NO: 61 - DNA, 291 bp, Artificial Sequence
  F49OncoRNA
taatacgactcactatagggataatacatttgcttctgacacaactgtgttcactagcaacctcaatggcggcccccggcagcgcccggcgacccctgctgctgctactgctgttgctgctgctcggcctcatgcattgtgcgtcagcagcaatggacgtgaacgagcaagtgtccctccgcggatcctacttcaccgcgaaggcgcatatgctggacatcatagaacttggaccgaaatcgtctgactacacaattgtgcttcctgtgattggggccatcgtggttggtc

SEQ ID NO: 62 - DNA, 291 bp, Artificial Sequence
  F50OncoRNA
taatacgactcactatagggataatacatttgcttctgacacaactgtgttcactagcaacctcaatggcggcccccggcagcgcccggcgacccctgctgctgctactgctgttgctgctgctcggcctcatgcattgtgcgtcagcagcaatggacttgccacaattgggtaaaatattcgggcgaatgaatactaaggcagatgcattgtctgagatagaggtgtatcactctgtttcgtctgactacacaattgtgcttcctgtgattggggccatcgtggttggtc

SEQ ID NO: 63 - DNA, 291 bp, Artificial Sequence
  F51OncoRNA
taatacgactcactatagggataatacatttgcttctgacacaactgtgttcactagcaacctcaatggcggcccccggcagcgcccggcgacccctgctgctgctactgctgttgctgctgctcggcctcatgcattgtgcgtcagcagcaatggacaaggaccgagcggaggctagcaagataccacaccttctccttgtaatgggtgagtttatcactcagtataatgtcggatcttcgtctgactacacaattgtgcttcctgtgattggggccatcgtggttggtc

SEQ ID NO: 64 - DNA, 291 bp, Artificial Sequence
  F52OncoRNA
taatacgactcactatagggataatacatttgcttctgacacaactgtgttcactagcaacctcaatggcggcccccggcagcgcccggcgacccctgctgctgctactgctgttgctgctgctcggcctcatgcattgtgcgtcagcagcaatggacgaaggtgtatttgagatgaaacgaaagggtatccaagcactcaacgcgtcagatccgcactacatacttgttttgacgagttcgtctgactacacaattgtgcttcctgtgattggggccatcgtggttggtc

SEQ ID NO: 65 - DNA, 291 bp, Artificial Sequence
  F53OncoRNA
taatacgactcactatagggataatacatttgcttctgacacaactgtgttcactagcaacctcaatggcggcccccggcagcgcccggcgacccctgctgctgctactgctgttgctgctgctcggcctcatgcattgtgcgtcagcagcaatggacatgaaactcggaaaagtacatgagcagtctccgcttataaaccttataacagcctcacgctttgcaggggactatgtggaatcgtctgactacacaattgtgcttcctgtgattggggccatcgtggttggtc

SEQ ID NO: 66 - DNA, 291 bp, Artificial Sequence
  F54OncoRNA
taatacgactcactatagggataatacatttgcttctgacacaactgtgttcactagcaacctcaatggcggcccccggcagcgcccggcgacccctgctgctgctactgctgttgctgctgctcggcctcatgcattgtgcgtcagcagcaatggacttgctccacataggggacctcaaaaagatgaactttcaggcaaggggcgctgttgagtacagtacatctgtcattgagccgtcgtctgactacacaattgtgcttcctgtgattggggccatcgtggttggtc

SEQ ID NO: 67 - DNA, 291 bp, Artificial Sequence
  F55OncoRNA
taatacgactcactatagggataatacatttgcttctgacacaactgtgttcactagcaacctcaatggcggcccccggcagcgcccggcgacccctgctgctgctactgctgttgctgctgctcggcctcatgcattgtgcgtcagcagcaatggacaaacactttcgaatacccgtggccaacaccggaggggacgtgctgctttctgagaagatgagtgcgtatgagctcattcaatcgtctgactacacaattgtgcttcctgtgattggggccatcgtggttggtc

SEQ ID NO: 68 - DNA, 291 bp, Artificial Sequence
  F56OncoRNA
taatacgactcactatagggataatacatttgcttctgacacaactgtgttcactagcaacctcaatggcggcccccggcagcgcccggcgacccctgctgctgctactgctgttgctgctgctcggcctcatgcattgtgcgtcagcagcaatggacctgtataagatgaggaagctggacgaggctgaactgtttatcggcggtataacgaacccatccgccgtgcatgtacagagctcgtctgactacacaattgtgcttcctgtgattggggccatcgtggttggtc

SEQ ID NO: 69 - DNA, 291 bp, Artificial Sequence
  F57OncoRNA
taatacgactcactatagggataatacatttgcttctgacacaactgtgttcactagcaacctcaatggcggcccccggcagcgcccggcgacccctgctgctgctactgctgttgctgctgctcggcctcatgcattgtgcgtcagcagcaatggacctgaatattgtatacccccagatgcgcaaaatagaggatgcgaagacctctttgagcgaggcgtttctggggggacacgtctcgtctgactacacaattgtgcttcctgtgattggggccatcgtggttggtc

SEQ ID NO: 70 - DNA, 291 bp, Artificial Sequence
  F58OncoRNA
taatacgactcactatagggataatacatttgcttctgacacaactgtgttcactagcaacctcaatggcggcccccggcagcgcccggcgacccctgctgctgctactgctgttgctgctgctcggcctcatgcattgtgcgtcagcagcaatggacgggaaggaagagatcatcttgtcttcagataacggatatgctttcaaaaggttgcatatgcctcaactcgtaacagtggcatcgtctgactacacaattgtgcttcctgtgattggggccatcgtggttggtc

SEQ ID NO: 71 - DNA, 291 bp, Artificial Sequence
  F59OncoRNA
taatacgactcactatagggataatacatttgcttctgacacaactgtgttcactagcaacctcaatggcggcccccggcagcgcccggcgacccctgctgctgctactgctgttgctgctgctcggcctcatgcattgtgcgtcagcagcaatggacgatttcagtgagggaggattgtataacgctcagaaagagaaaccacttgcagtgattcttcatagggtgatgtctacaatctcgtctgactacacaattgtgcttcctgtgattggggccatcgtggttggtc

SEQ ID NO: 72 - DNA, 291 bp, Artificial Sequence
  F60OncoRNA
taatacgactcactatagggataatacatttgcttctgacacaactgtgttcactagcaacctcaatggcggcccccggcagcgcccggcgacccctgctgctgctactgctgttgctgctgctcggcctcatgcattgtgcgtcagcagcaatggactcccacgccaaggaggttgctacgggctcattgatccagtttagactgggtgagccgatggacatttataaggttcttaactcgtctgactacacaattgtgcttcctgtgattggggccatcgtggttggtc

SEQ ID NO: 73 - DNA, 18 bp, Artificial Sequence
  promoter sequence of SP6 RNA polymerase
atttaggtgacactatag

SEQ ID NO: 74 - DNA, 18 bp, artificial sequence
  promoter sequence of T3 RNA polymerase
aattaaccctcactaaag

SEQ ID NO: 75 - DNA, 15 bp, Artificial Sequence
  promoter sequence of Syn5 RNA polymerase
attgggcacccgtaa

SEQ ID NO: 76 - DNA, 16 bp, artificial sequence
  the promoter sequence of KP34 RNA polymerase (strong promotor 1)
taatgttacaggagta

SEQ ID NO: 77 - DNA, 16 bp, artificial sequence
  promoter sequence of KP34 RNA polymerase (strong promotor 2)
tgatgttacaggagta

SEQ ID NO: 78 - DNA, 20 bp, artificial sequence
  promoter sequence of KP34 RNA polymerase (weak promotor)
actttggacatccgtcaagt

SEQ ID NO: 79 - DNA, 102 bp, artificial sequence
  reverse primer having a sequence 5' (T100)-GC -3'
ttttttttttttttttttttttttttttttttttttttttttttttttttttttttttttttttttttttttttttttttttttttttttttttttttttgc

SEQ ID NO: 80 - DNA, 151 bp, Artificial sequence
  reverse primer having a sequence 5' (T120)-GCAATGAAAATAAATGTTTTTTATTAGGCAG -3' (R_Mk2_120T)
ttttttttttttttttttttttttttttttttttttttttttttttttttttttttttttttttttttttttttttttttttttttttttttttttttttttttttttttttttttttttgcaatgaaaataaatgttttttattaggcag